European Patent Application EP 4 134 133 A1, published February 15, 2023. Title: Pegylated tetanus neurotoxins and treatment of hypotonia. Applicant: Snoretox Pty Ltd. Application EP. The sequence listing filed with the application follows.

SEQUENCE LISTING (17 sequences)

SEQ ID NO: 1 - protein, 1314 aa, Escherichia coli
PITINNFRYSDPVNNDTIIMMEPPYCKGLDIYYKAFKITDRIWIVPERYEFGTKPEDFNPPSSLIEGASEYYDPNYLRTDSDKDRFLQTMVKLFNRIKNNVAGEALLDKIINAIPYLGNSYSLLDKFDTNSNSVSFNLLEQDPSGATTKSAMLTNLIIFGPGPVLNKNEVRGIVLRVDNKNYFPCRDGFGSIMQMAFCPEYVPTFDNVIENITSLTIGKSKYFQDPALLLMHELIHVLHGLYGMQVSSHEIIPSKQEIYMQHTYPISAEELFTFGGQDANLISIDIKNDLYEKTLNDYKAIANKLSQVTSCNDPNIDIDSYKQIYQQKYQFDKDSNGQYIVNEDKFQILYNSIMYGFTEIELGKKFNIKTRLSYFSMNHDPVKIPNLLDDTIYNDTEGFNIESKDLKSEYKGQNMRVNTNAFRNVDGSGLVSKLIGLCKKIIPPTNIRENLYNRTASLTDLGGELCIKIKNEDLTFIAEKNSFSEEPFQDEIVSYNTKNKPLNFNYSLDKIIVDYNLQSKITLPNDRTTPVTKGIPYAPEYKSNAASTIEIHNIDDNTIYQYLYAQKSPTTLQRITMTNSVDDALINSTKIYSYFPSVISKVNQGAQGILFLQWVRDIIDDFTNESSQKTTIDKISDVSTIVPYIGPALNIVKQGYEGNFIGALETTGVVLLLEYIPEITLPVIAALSIAESSTQKEKIIKTIDNFLEKRYEKWIEVYKLVKAKWLGTVNTQFQKRSYQMYRSLEYQVDAIKKIIDYEYKIYSGPDKEQIADEINNLKNKLEEKANKAMININIFMRESSRSFLVNQMINEAKKQLLEFDTQSKNILMQYIKANSKFIGITELKKLESKINKVFSTPIPFSYSKNLDCWVDNEEDIDVILKKSTILNLDINNDIISDISGFNSSVITYPDAQLVPGINGKAIHLVNNESSEVIVHKAMDIEYNDMFNNFTVSFWLRVPKVSASHLEQYGTNEYSIISSMKKHSLSIGSGWSVSLKGNNLIWTLKDSAGEVRQITFRDLPDKFNAYLANKWVFITITNDRLSSANLYINGVLMGSAEITGLGAIREDNNITLKLDRCNNNNQYVSIDKFRIFCKALNPKEIEKLYTSYLSITFLRDFWGNPLRYDTEYYLIPVASSSKDVQLKNITDYMYLTNAPSYTNGKLNIYYRRLYNGLKFIIKRYTPNNEIDSFVKSGDFIKLYVSYNNNEHIVGYPKDGNAFNNLDRILRVGYNAPGIPLYKKMEAVKLRDLKTYSVQLKLYDDKNASLGLVGTHNGQIGNDPNRDILIASNWYFNHLKDKILGCDWYFVPTDEGWTND

SEQ ID NO: 2 - DNA, 6816 bp, Escherichia coli
  source 1..6816: mol_type = other DNA
gatctcgatcccgcgaaattaatacgactcactatagggagaccacaacggtttccctctagaaataattttgtttaactttaagaaggagatatacatatgcggggttctcatcatcatcatcatcatggtatggctagcatgactggtggacagcaaatgggtcgggatctgtacgacgatgacgataaggatcgatggggatccgagctcgagccgattaccatcaataattttcgttattcagatccggtgaataatgataccatcatcatgatggaaccaccgtactgtaaagggctggatatttattataaagcgttcaaaatcaccgaccgcatctggatcgtgccggaacgctacgaattcggcaccaaaccggaagattttaatccgccgagtagtctgatcgaaggtgcatcggaatactacgatccgaattatctgcgtactgactctgataaagatcgctttctgcaaacgatggtaaaactgttcaatcgtatcaaaaacaatgtagcaggcgaagccctgctggataaaatcatcaacgccattccgtatctgggaaacagttattctctgctggataaattcgatacaaactcgaactctgtgtcattcaacctgctggaacaggacccgagcggcgcgaccactaagagtgcgatgctgactaacctgattattttcggtccgggaccggtactgaataaaaatgaagttcgcggcattgtactgcgtgtcgataataaaaactatttcccatgtcgtgatggcttcggcagcatcatgcagatggccttttgtccggaatatgtgccaactttcgataatgtgattgagaacatcacctctctgacgattggtaaaagtaaatatttccaggatccggctctgctgctgatgcatgaactgatccatgttctgcatggcctgtatggcatgcaggtttcatcccacgaaattatcccatccaaacaggaaatttacatgcagcatacatatccgattagtgccgaagaactgttcacttttggcggccaggatgcgaacctgatttcgattgacattaaaaacgatctgtatgaaaaaactctgaacgattataaagcgattgccaacaaactgtctcaggtaacctcctgtaacgatccgaatattgatattgacagttataaacaaatttatcagcagaagtatcagttcgataaagactctaatggccagtatattgttaacgaagataaattccagattctgtacaatagcattatgtatggctttactgagatcgaactgggtaaaaaatttaacatcaagactcgtctgagctattttagcatgaatcatgatccagtgaaaatcccgaatctgctggatgatacgatttataatgataccgaaggatttaacatcgaaagcaaggatctgaaatccgaatataaagggcagaacatgcgcgttaataccaatgcatttcgcaatgttgatggttcaggcctggtgtcgaaactgattgggctgtgtaagaaaatcattccaccgacaaatattcgcgaaaatctgtacaaccgtacggcgagcctgaccgatctggggggagaactgtgtattaaaatcaaaaatgaagatctgaccttcattgctgagaagaatagcttttccgaagagccattccaggacgaaatcgtgtcttataacaccaagaataaaccgctgaatttcaactactccctggacaaaatcattgtggattacaacctgcagagtaaaattaccctgccgaatgatcgtaccaccccggtgacgaaaggcatcccttacgcaccagaatataaatcaaatgcagcctcgactatcgagatccataatattgatgacaacactatttaccagtacctgtatgctcagaaatctccgacgacgctgcagcgcatcaccatgactaacagcgtggacgatgccctgattaatagcaccaaaatctactcttactttccgtcggtgatctctaaggttaatcagggcgcgcaaggtatcctgtttctgcaatgggtgcgtgatattattgatgatttcactaatgaatctagccagaaaacgacaattgataaaatttcggatgtttccaccatcgtgccttacatcggcccagcgctgaacatcgtgaagcagggttatgagggtaactttatcggagcactggaaacgaccggcgtggttctgctgctggaatatattccggagattactctgccagttattgcggctctgtcgattgcagagagctcaacgcagaaagaaaaaattattaagacgatcgacaatttcctggaaaagcgctacgaaaaatggatcgaagtgtataagctggtgaaagcgaaatggctggggaccgtgaacacccagttccaaaaacgttcctatcaaatgtatcgtagcctggaatatcaggtggacgccattaaaaagatcatcgattacgaatataagatctactccggtccggacaaagaacagattgcggacgaaattaacaatctgaaaaataaactggaggaaaaagccaacaaagcgatgattaatatcaatattttcatgcgtgaaagcagccgtagcttcctggtcaatcagatgattaatgaagcgaagaaacaactgctggaatttgatacgcaatctaaaaatattctgatgcaatacatcaaagccaattctaaatttattgggatcacggaactgaaaaagctggaatcgaaaatcaataaagtctttagcaccccgattccgttctcctactcgaaaaatctggattgttgggttgacaatgaagaagatattgatgttattctgaaaaagagcacgatcctgaacctggatattaataacgatattatctctgatatcagtggttttaattcatcagttattacttacccagacgctcaactggtgccgggaatcaatgggaaagccattcatctggtgaataatgaatcaagtgaagtgatcgtgcataaagcgatggatatcgagtacaacgatatgtttaataatttcacggtgtcgttctggctgcgtgttccgaaagtgagtgcctcccacctggaacaatatggaaccaacgaatactcaatcattagcagcatgaagaaacattcgctgagtattggttcaggttggagcgtttccctgaaagggaacaatctgatctggacactgaaggactcagcgggcgaagtgcgtcagattacgtttcgtgatctgccggataaatttaatgcatacctggctaacaaatgggtgttcatcacaatcaccaatgaccgtctgtcgtctgcaaacctgtatattaatggggtactgatgggctcggcagaaattacagggctgggcgccattcgtgaagataacaatattacgctgaaactggatcgttgtaataacaataatcagtatgtgagcattgataaatttcgtattttctgcaaagcgctgaacccgaaagaaattgaaaaactgtatacctcgtatctgtcaattacgtttctgcgcgatttctggggaaacccgctgcgttacgatacggaatactacctgatcccggtagccagttctagtaaagacgttcaactgaaaaatattaccgactacatgtatctgacaaacgctccatcatacacaaacggcaaactgaacatctattaccgtcgcctgtacaatgggctgaaattcatcattaaacgttataccccgaataacgaaattgattcctttgtgaagtccggtgacttcattaagctgtatgtatcctataacaataatgaacacatcgttggctatccgaaggatggcaatgcctttaacaacctggatcgtattctgcgtgtaggttacaacgccccgggtattccgctgtataagaaaatggaagcagtgaaactgcgtgatctgaaaacatattccgtgcaactgaagctgtatgatgacaaaaatgctagcctgggtctggtaggcacgcataacggtcagattggaaacgatcctaatcgtgacatcctgatcgcctctaactggtattttaaccacctgaaagataaaattctgggctgcgattggtattttgtccctaccgatgaaggctggacgaacgattaaaagcttgatccggctgctaacaaagcccgaaaggaagctgagttggctgctgccaccgctgagcaataactagcataaccccttggggcctctaaacgggtcttgaggggttttttgctgaaaggaggaactatatccggatctggcgtaatagcgaagaggcccgcaccgatcgcccttcccaacagttgcgcagcctgaatggcgaatgggacgcgccctgtagcggcgcattaagcgcggcgggtgtggtggttacgcgcagcgtgaccgctacacttgccagcgccctagcgcccgctcctttcgctttcttcccttcctttctcgccacgttcgccggctttccccgtcaagctctaaatcgggggctccctttagggttccgatttagtgctttacggcacctcgaccccaaaaaacttgattagggtgatggttcacgtagtgggccatcgccctgatagacggtttttcgccctttgacgttggagtccacgttctttaatagtggactcttgttccaaactggaacaacactcaaccctatctcggtctattcttttgatttataagggattttgccgatttcggcctattggttaaaaaatgagctgatttaacaaaaatttaacgcgaattttaacaaaatattaacgcttacaatttaggtggcacttttcggggaaatgtgcgcggaacccctatttgtttatttttctaaatacattcaaatatgtatccgctcatgagacaataaccctgataaatgcttcaataatattgaaaaaggaagagtatgagtattcaacatttccgtgtcgcccttattcccttttttgcggcattttgccttcctgtttttgctcacccagaaacgctggtgaaagtaaaagatgctgaagatcagttgggtgcacgagtgggttacatcgaactggatctcaacagcggtaagatccttgagagttttcgccccgaagaacgttttccaatgatgagcacttttaaagttctgctatgtggcgcggtattatcccgtattgacgccgggcaagagcaactcggtcgccgcatacactattctcagaatgacttggttgagtactcaccagtcacagaaaagcatcttacggatggcatgacagtaagagaattatgcagtgctgccataaccatgagtgataacactgcggccaacttacttctgacaacgatcggaggaccgaaggagctaaccgcttttttgcacaacatgggggatcatgtaactcgccttgatcgttgggaaccggagctgaatgaagccataccaaacgacgagcgtgacaccacgatgcctgtagcaatggcaacaacgttgcgcaaactattaactggcgaactacttactctagcttcccggcaacaattaatagactggatggaggcggataaagttgcaggaccacttctgcgctcggcccttccggctggctggtttattgctgataaatctggagccggtgagcgtgggtctcgcggtatcattgcagcactggggccagatggtaagccctcccgtatcgtagttatctacacgacggggagtcaggcaactatggatgaacgaaatagacagatcgctgagataggtgcctcactgattaagcattggtaactgtcagaccaagtttactcatatatactttagattgatttaaaacttcatttttaatttaaaaggatctaggtgaagatcctttttgataatctcatgaccaaaatcccttaacgtgagttttcgttccactgagcgtcagaccccgtagaaaagatcaaaggatcttcttgagatcctttttttctgcgcgtaatctgctgcttgcaaacaaaaaaaccaccgctaccagcggtggtttgtttgccggatcaagagctaccaactctttttccgaaggtaactggcttcagcagagcgcagataccaaatactgttcttctagtgtagccgtagttaggccaccacttcaagaactctgtagcaccgcctacatacctcgctctgctaatcctgttaccagtggctgctgccagtggcgataagtcgtgtcttaccgggttggactcaagacgatagttaccggataaggcgcagcggtcgggctgaacggggggttcgtgcacacagcccagcttggagcgaacgacctacaccgaactgagatacctacagcgtgagctatgagaaagcgccacgcttcccgaagggagaaaggcggacaggtatccggtaagcggcagggtcggaacaggagagcgcacgagggagcttccagggggaaacgcctggtatctttatagtcctgtcgggtttcgccacctctgacttgagcgtcgatttttgtgatgctcgtcaggggggcggagcctatggaaaaacgccagcaacgcggcctttttacggttcctggccttttgctggccttttgctcacatgttctttcctgcgttatcccctgattctgtggataaccgtattaccgcctttgagtgagctgataccgctcgccgcagccgaacgaccgagcgcagcgagtcagtgagcgaggaagcggaagagcgcccaatacgcaaaccgcctctccccgcgcgttggccgattcattaatgcag

SEQ ID NO: 3 - protein, 858 aa, Escherichia coli
SLTDLGGELCIKIKNEDLTFIAEKNSFSEEPFQDEIVSYNTKNKPLNFNYSLDKIIVDYNLQSKITLPNDRTTPVTKGIPYAPEYKSNAASTIEIHNIDDNTIYQYLYAQKSPTTLQRITMTNSVDDALINSTKIYSYFPSVISKVNQGAQGILFLQWVRDIIDDFTNESSQKTTIDKISDVSTIVPYIGPALNIVKQGYEGNFIGALETTGVVLLLEYIPEITLPVIAALSIAESSTQKEKIIKTIDNFLEKRYEKWIEVYKLVKAKWLGTVNTQFQKRSYQMYRSLEYQVDAIKKIIDYEYKIYSGPDKEQIADEINNLKNKLEEKANKAMININIFMRESSRSFLVNQMINEAKKQLLEFDTQSKNILMQYIKANSKFIGITELKKLESKINKVFSTPIPFSYSKNLDCWVDNEEDIDVILKKSTILNLDINNDIISDISGFNSSVITYPDAQLVPGINGKAIHLVNNESSEVIVHKAMDIEYNDMFNNFTVSFWLRVPKVSASHLEQYGTNEYSIISSMKKHSLSIGSGWSVSLKGNNLIWTLKDSAGEVRQITFRDLPDKFNAYLANKWVFITITNDRLSSANLYINGVLMGSAEITGLGAIREDNNITLKLDRCNNNNQYVSIDKFRIFCKALNPKEIEKLYTSYLSITFLRDFWGNPLRYDTEYYLIPVASSSKDVQLKNITDYMYLTNAPSYTNGKLNIYYRRLYNGLKFIIKRYTPNNEIDSFVKSGDFIKLYVSYNNNEHIVGYPKDGNAFNNLDRILRVGYNAPGIPLYKKMEAVKLRDLKTYSVQLKLYDDKNASLGLVGTHNGQIGNDPNRDILIASNWYFNHLKDKILGCDWYFVPTDEGWTND

SEQ ID NO: 4 - protein, 451 aa, Escherichia coli
KNLDCWVDNEEDIDVILKKSTILNLDINNDIISDISGFNSSVITYPDAQLVPGINGKAIHLVNNESSEVIVHKAMDIEYNDMFNNFTVSFWLRVPKVSASHLEQYGTNEYSIISSMKKHSLSIGSGWSVSLKGNNLIWTLKDSAGEVRQITFRDLPDKFNAYLANKWVFITITNDRLSSANLYINGVLMGSAEITGLGAIREDNNITLKLDRCNNNNQYVSIDKFRIFCKALNPKEIEKLYTSYLSITFLRDFWGNPLRYDTEYYLIPVASSSKDVQLKNITDYMYLTNAPSYTNGKLNIYYRRLYNGLKFIIKRYTPNNEIDSFVKSGDFIKLYVSYNNNEHIVGYPKDGNAFNNLDRILRVGYNAPGIPLYKKMEAVKLRDLKTYSVQLKLYDDKNASLGLVGTHNGQIGNDPNRDILIASNWYFNHLKDKILGCDWYFVPTDEGWTND

SEQ ID NO: 5 - DNA, 4234 bp, Escherichia coli
  source 1..4234: mol_type = other DNA
gatctcgatcccgcgaaattaatacgactcactatagggagaccacaacggtttccctctagaaataattttgtttaactttaagaaggagatatacatatgcggggttctcatcatcatcatcatcatggtatggctagcatgactggtggacagcaaatgggtcgggatctgtacgacgatgacgataaggatcgatggggatccgagctcgagaaaaatctggattgttgggttgacaatgaagaagatattgatgttattctgaaaaagagcacgatcctgaacctggatattaataacgatattatctctgatatcagtggttttaattcatcagttattacttacccagacgctcaactggtgccgggaatcaatgggaaagccattcatctggtgaataatgaatcaagtgaagtgatcgtgcataaagcgatggatatcgagtacaacgatatgtttaataatttcacggtgtcgttctggctgcgtgttccgaaagtgagtgcctcccacctggaacaatatggaaccaacgaatactcaatcattagcagcatgaagaaacattcgctgagtattggttcaggttggagcgtttccctgaaagggaacaatctgatctggacactgaaggactcagcgggcgaagtgcgtcagattacgtttcgtgatctgccggataaatttaatgcatacctggctaacaaatgggtgttcatcacaatcaccaatgaccgtctgtcgtctgcaaacctgtatattaatggggtactgatgggctcggcagaaattacagggctgggcgccattcgtgaagataacaatattacgctgaaactggatcgttgtaataacaataatcagtatgtgagcattgataaatttcgtattttctgcaaagcgctgaacccgaaagaaattgaaaaactgtatacctcgtatctgtcaattacgtttctgcgcgatttctggggaaacccgctgcgttacgatacggaatactacctgatcccggtagccagttctagtaaagacgttcaactgaaaaatattaccgactacatgtatctgacaaacgctccatcatacacaaacggcaaactgaacatctattaccgtcgcctgtacaatgggctgaaattcatcattaaacgttataccccgaataacgaaattgattcctttgtgaagtccggtgacttcattaagctgtatgtatcctataacaataatgaacacatcgttggctatccgaaggatggcaatgcctttaacaacctggatcgtattctgcgtgtaggttacaacgccccgggtattccgctgtataagaaaatggaagcagtgaaactgcgtgatctgaaaacatattccgtgcaactgaagctgtatgatgacaaaaatgctagcctgggtctggtaggcacgcataacggtcagattggaaacgatcctaatcgtgacatcctgatcgcctctaactggtattttaaccacctgaaagataaaattctgggctgcgattggtattttgtccctaccgatgaaggctggacgaacgattaagaattcgaagcttgatccggctgctaacaaagcccgaaaggaagctgagttggctgctgccaccgctgagcaataactagcataaccccttggggcctctaaacgggtcttgaggggttttttgctgaaaggaggaactatatccggatctggcgtaatagcgaagaggcccgcaccgatcgcccttcccaacagttgcgcagcctgaatggcgaatgggacgcgccctgtagcggcgcattaagcgcggcgggtgtggtggttacgcgcagcgtgaccgctacacttgccagcgccctagcgcccgctcctttcgctttcttcccttcctttctcgccacgttcgccggctttccccgtcaagctctaaatcgggggctccctttagggttccgatttagtgctttacggcacctcgaccccaaaaaacttgattagggtgatggttcacgtagtgggccatcgccctgatagacggtttttcgccctttgacgttggagtccacgttctttaatagtggactcttgttccaaactggaacaacactcaaccctatctcggtctattcttttgatttataagggattttgccgatttcggcctattggttaaaaaatgagctgatttaacaaaaatttaacgcgaattttaacaaaatattaacgcttacaatttaggtggcacttttcggggaaatgtgcgcggaacccctatttgtttatttttctaaatacattcaaatatgtatccgctcatgagacaataaccctgataaatgcttcaataatattgaaaaaggaagagtatgagtattcaacatttccgtgtcgcccttattcccttttttgcggcattttgccttcctgtttttgctcacccagaaacgctggtgaaagtaaaagatgctgaagatcagttgggtgcacgagtgggttacatcgaactggatctcaacagcggtaagatccttgagagttttcgccccgaagaacgttttccaatgatgagcacttttaaagttctgctatgtggcgcggtattatcccgtattgacgccgggcaagagcaactcggtcgccgcatacactattctcagaatgacttggttgagtactcaccagtcacagaaaagcatcttacggatggcatgacagtaagagaattatgcagtgctgccataaccatgagtgataacactgcggccaacttacttctgacaacgatcggaggaccgaaggagctaaccgcttttttgcacaacatgggggatcatgtaactcgccttgatcgttgggaaccggagctgaatgaagccataccaaacgacgagcgtgacaccacgatgcctgtagcaatggcaacaacgttgcgcaaactattaactggcgaactacttactctagcttcccggcaacaattaatagactggatggaggcggataaagttgcaggaccacttctgcgctcggcccttccggctggctggtttattgctgataaatctggagccggtgagcgtgggtctcgcggtatcattgcagcactggggccagatggtaagccctcccgtatcgtagttatctacacgacggggagtcaggcaactatggatgaacgaaatagacagatcgctgagataggtgcctcactgattaagcattggtaactgtcagaccaagtttactcatatatactttagattgatttaaaacttcatttttaatttaaaaggatctaggtgaagatcctttttgataatctcatgaccaaaatcccttaacgtgagttttcgttccactgagcgtcagaccccgtagaaaagatcaaaggatcttcttgagatcctttttttctgcgcgtaatctgctgcttgcaaacaaaaaaaccaccgctaccagcggtggtttgtttgccggatcaagagctaccaactctttttccgaaggtaactggcttcagcagagcgcagataccaaatactgttcttctagtgtagccgtagttaggccaccacttcaagaactctgtagcaccgcctacatacctcgctctgctaatcctgttaccagtggctgctgccagtggcgataagtcgtgtcttaccgggttggactcaagacgatagttaccggataaggcgcagcggtcgggctgaacggggggttcgtgcacacagcccagcttggagcgaacgacctacaccgaactgagatacctacagcgtgagctatgagaaagcgccacgcttcccgaagggagaaaggcggacaggtatccggtaagcggcagggtcggaacaggagagcgcacgagggagcttccagggggaaacgcctggtatctttatagtcctgtcgggtttcgccacctctgacttgagcgtcgatttttgtgatgctcgtcaggggggcggagcctatggaaaaacgccagcaacgcggcctttttacggttcctggccttttgctggccttttgctcacatgttctttcctgcgttatcccctgattctgtggataaccgtattaccgcctttgagtgagctgataccgctcgccgcagccgaacgaccgagcgcagcgagtcagtgagcgaggaagcggaagagcgcccaatacgcaaaccgcctctccccgcgcgttggccgattcattaatgcag

SEQ ID NO: 6 - protein, 863 aa, Escherichia coli
PITINNFRYSDPVNNDTIIMMEPPYCKGLDIYYKAFKITDRIWIVPERYEFGTKPEDFNPPSSLIEGASEYYDPNYLRTDSDKDRFLQTMVKLFNRIKNNVAGEALLDKIINAIPYLGNSYSLLDKFDTNSNSVSFNLLEQDPSGATTKSAMLTNLIIFGPGPVLNKNEVRGIVLRVDNKNYFPCRDGFGSIMQMAFCPEYVPTFDNVIENITSLTIGKSKYFQDPALLLMHELIHVLHGLYGMQVSSHEIIPSKQEIYMQHTYPISAEELFTFGGQDANLISIDIKNDLYEKTLNDYKAIANKLSQVTSCNDPNIDIDSYKQIYQQKYQFDKDSNGQYIVNEDKFQILYNSIMYGFTEIELGKKFNIKTRLSYFSMNHDPVKIPNLLDDTIYNDTEGFNIESKDLKSEYKGQNMRVNTNAFRNVDGSGLVSKLIGLCKKIIPPTNIRENLYNRTASLTDLGGELCIKIKNEDLTFIAEKNSFSEEPFQDEIVSYNTKNKPLNFNYSLDKIIVDYNLQSKITLPNDRTTPVTKGIPYAPEYKSNAASTIEIHNIDDNTIYQYLYAQKSPTTLQRITMTNSVDDALINSTKIYSYFPSVISKVNQGAQGILFLQWVRDIIDDFTNESSQKTTIDKISDVSTIVPYIGPALNIVKQGYEGNFIGALETTGVVLLLEYIPEITLPVIAALSIAESSTQKEKIIKTIDNFLEKRYEKWIEVYKLVKAKWLGTVNTQFQKRSYQMYRSLEYQVDAIKKIIDYEYKIYSGPDKEQIADEINNLKNKLEEKANKAMININIFMRESSRSFLVNQMINEAKKQLLEFDTQSKNILMQYIKANSKFIGITELKKLESKINKVFSTPIPFSYS

SEQ ID NO: 7 - DNA, 5479 bp, Escherichia coli
  source 1..5479: mol_type = other DNA
gatctcgatcccgcgaaattaatacgactcactatagggagaccacaacggtttccctctagaaataattttgtttaactttaagaaggagatatacatatgcggggttctcatcatcatcatcatcatggtatggctagcatgactggtggacagcaaatgggtcgggatctgtacgacgatgacgataaggatcgatggggatccgagctcgagccgattaccatcaataattttcgttattcagatccggtgaataatgataccatcatcatgatggaaccaccgtactgtaaagggctggatatttattataaagcgttcaaaatcaccgaccgcatctggatcgtgccggaacgctacgaattcggcaccaaaccggaagattttaatccgccgagtagtctgatcgaaggtgcatcggaatactacgatccgaattatctgcgtactgactctgataaagatcgctttctgcaaacgatggtaaaactgttcaatcgtatcaaaaacaatgtagcaggcgaagccctgctggataaaatcatcaacgccattccgtatctgggaaacagttattctctgctggataaattcgatacaaactcgaactctgtgtcattcaacctgctggaacaggacccgagcggcgcgaccactaagagtgcgatgctgactaacctgattattttcggtccgggaccggtactgaataaaaatgaagttcgcggcattgtactgcgtgtcgataataaaaactatttcccatgtcgtgatggcttcggcagcatcatgcagatggccttttgtccggaatatgtgccaactttcgataatgtgattgagaacatcacctctctgacgattggtaaaagtaaatatttccaggatccggctctgctgctgatgcatgaactgatccatgttctgcatggcctgtatggcatgcaggtttcatcccacgaaattatcccatccaaacaggaaatttacatgcagcatacatatccgattagtgccgaagaactgttcacttttggcggccaggatgcgaacctgatttcgattgacattaaaaacgatctgtatgaaaaaactctgaacgattataaagcgattgccaacaaactgtctcaggtaacctcctgtaacgatccgaatattgatattgacagttataaacaaatttatcagcagaagtatcagttcgataaagactctaatggccagtatattgttaacgaagataaattccagattctgtacaatagcattatgtatggctttactgagatcgaactgggtaaaaaatttaacatcaagactcgtctgagctattttagcatgaatcatgatccagtgaaaatcccgaatctgctggatgatacgatttataatgataccgaaggatttaacatcgaaagcaaggatctgaaatccgaatataaagggcagaacatgcgcgttaataccaatgcatttcgcaatgttgatggttcaggcctggtgtcgaaactgattgggctgtgtaagaaaatcattccaccgacaaatattcgcgaaaatctgtacaaccgtacggcgagcctgaccgatctggggggagaactgtgtattaaaatcaaaaatgaagatctgaccttcattgctgagaagaatagcttttccgaagagccattccaggacgaaatcgtgtcttataacaccaagaataaaccgctgaatttcaactactccctggacaaaatcattgtggattacaacctgcagagtaaaattaccctgccgaatgatcgtaccaccccggtgacgaaaggcatcccttacgcaccagaatataaatcaaatgcagcctcgactatcgagatccataatattgatgacaacactatttaccagtacctgtatgctcagaaatctccgacgacgctgcagcgcatcaccatgactaacagcgtggacgatgccctgattaatagcaccaaaatctactcttactttccgtcggtgatctctaaggttaatcagggcgcgcaaggtatcctgtttctgcaatgggtgcgtgatattattgatgatttcactaatgaatctagccagaaaacgacaattgataaaatttcggatgtttccaccatcgtgccttacatcggcccagcgctgaacatcgtgaagcagggttatgagggtaactttatcggagcactggaaacgaccggcgtggttctgctgctggaatatattccggagattactctgccagttattgcggctctgtcgattgcagagagctcaacgcagaaagaaaaaattattaagacgatcgacaatttcctggaaaagcgctacgaaaaatggatcgaagtgtataagctggtgaaagcgaaatggctggggaccgtgaacacccagttccaaaaacgttcctatcaaatgtatcgtagcctggaatatcaggtggacgccattaaaaagatcatcgattacgaatataagatctactccggtccggacaaagaacagattgcggacgaaattaacaatctgaaaaataaactggaggaaaaagccaacaaagcgatgattaatatcaatattttcatgcgtgaaagcagccgtagcttcctggtcaatcagatgattaatgaagcgaagaaacaactgctggaatttgatacgcaatctaaaaatattctgatgcaatacatcaaagccaattctaaatttattgggatcacggaactgaaaaagctggaatcgaaaatcaataaagtctttagcaccccgattccgttctcctactcgtaaggtaccatggaattcgaagcttgatccggctgctaacaaagcccgaaaggaagctgagttggctgctgccaccgctgagcaataactagcataaccccttggggcctctaaacgggtcttgaggggttttttgctgaaaggaggaactatatccggatctggcgtaatagcgaagaggcccgcaccgatcgcccttcccaacagttgcgcagcctgaatggcgaatgggacgcgccctgtagcggcgcattaagcgcggcgggtgtggtggttacgcgcagcgtgaccgctacacttgccagcgccctagcgcccgctcctttcgctttcttcccttcctttctcgccacgttcgccggctttccccgtcaagctctaaatcgggggctccctttagggttccgatttagtgctttacggcacctcgaccccaaaaaacttgattagggtgatggttcacgtagtgggccatcgccctgatagacggtttttcgccctttgacgttggagtccacgttctttaatagtggactcttgttccaaactggaacaacactcaaccctatctcggtctattcttttgatttataagggattttgccgatttcggcctattggttaaaaaatgagctgatttaacaaaaatttaacgcgaattttaacaaaatattaacgcttacaatttaggtggcacttttcggggaaatgtgcgcggaacccctatttgtttatttttctaaatacattcaaatatgtatccgctcatgagacaataaccctgataaatgcttcaataatattgaaaaaggaagagtatgagtattcaacatttccgtgtcgcccttattcccttttttgcggcattttgccttcctgtttttgctcacccagaaacgctggtgaaagtaaaagatgctgaagatcagttgggtgcacgagtgggttacatcgaactggatctcaacagcggtaagatccttgagagttttcgccccgaagaacgttttccaatgatgagcacttttaaagttctgctatgtggcgcggtattatcccgtattgacgccgggcaagagcaactcggtcgccgcatacactattctcagaatgacttggttgagtactcaccagtcacagaaaagcatcttacggatggcatgacagtaagagaattatgcagtgctgccataaccatgagtgataacactgcggccaacttacttctgacaacgatcggaggaccgaaggagctaaccgcttttttgcacaacatgggggatcatgtaactcgccttgatcgttgggaaccggagctgaatgaagccataccaaacgacgagcgtgacaccacgatgcctgtagcaatggcaacaacgttgcgcaaactattaactggcgaactacttactctagcttcccggcaacaattaatagactggatggaggcggataaagttgcaggaccacttctgcgctcggcccttccggctggctggtttattgctgataaatctggagccggtgagcgtgggtctcgcggtatcattgcagcactggggccagatggtaagccctcccgtatcgtagttatctacacgacggggagtcaggcaactatggatgaacgaaatagacagatcgctgagataggtgcctcactgattaagcattggtaactgtcagaccaagtttactcatatatactttagattgatttaaaacttcatttttaatttaaaaggatctaggtgaagatcctttttgataatctcatgaccaaaatcccttaacgtgagttttcgttccactgagcgtcagaccccgtagaaaagatcaaaggatcttcttgagatcctttttttctgcgcgtaatctgctgcttgcaaacaaaaaaaccaccgctaccagcggtggtttgtttgccggatcaagagctaccaactctttttccgaaggtaactggcttcagcagagcgcagataccaaatactgttcttctagtgtagccgtagttaggccaccacttcaagaactctgtagcaccgcctacatacctcgctctgctaatcctgttaccagtggctgctgccagtggcgataagtcgtgtcttaccgggttggactcaagacgatagttaccggataaggcgcagcggtcgggctgaacggggggttcgtgcacacagcccagcttggagcgaacgacctacaccgaactgagatacctacagcgtgagctatgagaaagcgccacgcttcccgaagggagaaaggcggacaggtatccggtaagcggcagggtcggaacaggagagcgcacgagggagcttccagggggaaacgcctggtatctttatagtcctgtcgggtttcgccacctctgacttgagcgtcgatttttgtgatgctcgtcaggggggcggagcctatggaaaaacgccagcaacgcggcctttttacggttcctggccttttgctggccttttgctcacatgttctttcctgcgttatcccctgattctgtggataaccgtattaccgcctttgagtgagctgataccgctcgccgcagccgaacgaccgagcgcagcgagtcagtgagcgaggaagcggaagagcgcccaatacgcaaaccgcctctccccgcgcgttggccgattcattaatgcag

SEQ ID NO: 8 - protein, 451 aa, Escherichia coli
KNLDCWVDNEEDIDVILKKSTILNLDINNDIISDISGFNSSVITYPDAQLVPGINGKAIHLVNNESSEVIVHKAMDIEYNDMFNNFTVSFWLRVPKVSASHLEQYGTNEYSIISSMKKHSLSIGSGWSVSLKGNNLIWTLKDSAGEVRQITFRDLPDKFNAYLANKWVFITITNDRLSSANLYINGVLMGSAEITGLGAIREDNNITLKLDRCNNNNQYVSIDKFRIFCKALNPKEIEKLYTSYLSITFLRDFWGNPLRYDTEYYLIPVASSSKDVQLKNITDYMYLTNAPSYTNGKLNIYYRRLYNGLKFIIKRYTPNNEIDSFVKSGDFIKLYVSYNNNEHIVGYPKDGNAFNNLDRILEVGYNAPGIPLYKKMEAVKLRDLKTYSVQLKLYDDKNASLGLVGTHNGQIGNDPNRDILIASNAYFNHLKDKILGCDWYFVPTDEGWTND

SEQ ID NO: 9 - DNA, 4234 bp, Escherichia coli
  source 1..4234: mol_type = other DNA
gatctcgatcccgcgaaattaatacgactcactatagggagaccacaacggtttccctctagaaataattttgtttaactttaagaaggagatatacatatgcggggttctcatcatcatcatcatcatggtatggctagcatgactggtggacagcaaatgggtcgggatctgtacgacgatgacgataaggatcgatggggatccgagctcgagaaaaatttggattgctgggtcgacaatgaggaggacattgatgtgatattaaagaaatccactatcttaaatcttgatataaacaatgacatcatctcggatatatctgggttcaattcttccgtcataacttaccctgatgctcaactggtaccgggaattaatgggaaggccatacacttagtcaacaacgaatcttccgaggtgattgtacataaggcaatggacatagagtacaatgacatgtttaataactttactgtctcgttctggttacgcgtgcccaaagtatctgcctcacacctggaacagtatggcacaaatgaatattctattatcagtagtatgaagaaacactcgctttctataggatccggctggagtgtttcgctgaagggcaataacttgatctggacccttaaagattcagcgggagaagtaagacaaataactttccgggatttgcctgataagttcaacgcatacctggccaataagtgggttttcataactataacaaatgaccgcttgtctagcgccaacttatacatcaatggagtattgatgggttccgctgagattacaggcttgggtgccataagagaggacaataatatcaccctgaaactggaccgctgcaataataacaatcagtacgtgagcatagataaattccgtattttttgcaaagccctgaacccgaaagaaatcgaaaaactgtatacttcatatctgagcataacatttctgcgtgatttttggggtaacccgctgcgttatgataccgaatactacctgattccggttgccagcagcagcaaagatgttcagctgaaaaatattaccgactatatgtatctgacaaatgcgccgtcttataccaatggcaaactgaatatttattatcgccggttgtacaacgggctgaagttcattattaaacggtacaccccgaacaacgaaatcgattcatttgttaaatccggggatttcataaagttatacgtgagctataataacaacgagcatattgtaggttatccgaaagacggtaatgctttcaacaacttggatcggatactggaagttggttacaacgccccaggtattccactgtataagaaaatggaagccgtcaagttgcgtgatttaaagacgtactcagtacagcttaaattatacgacgataagaatgcaagccttggattggttgggacccacaatggtcagattggaaatgaccccaatcgggacattctgatagcatccaacgcgtacttcaaccatttgaaagataaaatcctgggctgtgattggtactttgtaccgactgatgaaggatggacgaatgactaagaattcgaagcttgatccggctgctaacaaagcccgaaaggaagctgagttggctgctgccaccgctgagcaataactagcataaccccttggggcctctaaacgggtcttgaggggttttttgctgaaaggaggaactatatccggatctggcgtaatagcgaagaggcccgcaccgatcgcccttcccaacagttgcgcagcctgaatggcgaatgggacgcgccctgtagcggcgcattaagcgcggcgggtgtggtggttacgcgcagcgtgaccgctacacttgccagcgccctagcgcccgctcctttcgctttcttcccttcctttctcgccacgttcgccggctttccccgtcaagctctaaatcgggggctccctttagggttccgatttagtgctttacggcacctcgaccccaaaaaacttgattagggtgatggttcacgtagtgggccatcgccctgatagacggtttttcgccctttgacgttggagtccacgttctttaatagtggactcttgttccaaactggaacaacactcaaccctatctcggtctattcttttgatttataagggattttgccgatttcggcctattggttaaaaaatgagctgatttaacaaaaatttaacgcgaattttaacaaaatattaacgcttacaatttaggtggcacttttcggggaaatgtgcgcggaacccctatttgtttatttttctaaatacattcaaatatgtatccgctcatgagacaataaccctgataaatgcttcaataatattgaaaaaggaagagtatgagtattcaacatttccgtgtcgcccttattcccttttttgcggcattttgccttcctgtttttgctcacccagaaacgctggtgaaagtaaaagatgctgaagatcagttgggtgcacgagtgggttacatcgaactggatctcaacagcggtaagatccttgagagttttcgccccgaagaacgttttccaatgatgagcacttttaaagttctgctatgtggcgcggtattatcccgtattgacgccgggcaagagcaactcggtcgccgcatacactattctcagaatgacttggttgagtactcaccagtcacagaaaagcatcttacggatggcatgacagtaagagaattatgcagtgctgccataaccatgagtgataacactgcggccaacttacttctgacaacgatcggaggaccgaaggagctaaccgcttttttgcacaacatgggggatcatgtaactcgccttgatcgttgggaaccggagctgaatgaagccataccaaacgacgagcgtgacaccacgatgcctgtagcaatggcaacaacgttgcgcaaactattaactggcgaactacttactctagcttcccggcaacaattaatagactggatggaggcggataaagttgcaggaccacttctgcgctcggcccttccggctggctggtttattgctgataaatctggagccggtgagcgtgggtctcgcggtatcattgcagcactggggccagatggtaagccctcccgtatcgtagttatctacacgacggggagtcaggcaactatggatgaacgaaatagacagatcgctgagataggtgcctcactgattaagcattggtaactgtcagaccaagtttactcatatatactttagattgatttaaaacttcatttttaatttaaaaggatctaggtgaagatcctttttgataatctcatgaccaaaatcccttaacgtgagttttcgttccactgagcgtcagaccccgtagaaaagatcaaaggatcttcttgagatcctttttttctgcgcgtaatctgctgcttgcaaacaaaaaaaccaccgctaccagcggtggtttgtttgccggatcaagagctaccaactctttttccgaaggtaactggcttcagcagagcgcagataccaaatactgttcttctagtgtagccgtagttaggccaccacttcaagaactctgtagcaccgcctacatacctcgctctgctaatcctgttaccagtggctgctgccagtggcgataagtcgtgtcttaccgggttggactcaagacgatagttaccggataaggcgcagcggtcgggctgaacggggggttcgtgcacacagcccagcttggagcgaacgacctacaccgaactgagatacctacagcgtgagctatgagaaagcgccacgcttcccgaagggagaaaggcggacaggtatccggtaagcggcagggtcggaacaggagagcgcacgagggagcttccagggggaaacgcctggtatctttatagtcctgtcgggtttcgccacctctgacttgagcgtcgatttttgtgatgctcgtcaggggggcggagcctatggaaaaacgccagcaacgcggcctttttacggttcctggccttttgctggccttttgctcacatgttctttcctgcgttatcccctgattctgtggataaccgtattaccgcctttgagtgagctgataccgctcgccgcagccgaacgaccgagcgcagcgagtcagtgagcgaggaagcggaagagcgcccaatacgcaaaccgcctctccccgcgcgttggccgattcattaatgcag

SEQ ID NO: 10 - protein, 1314 aa, Escherichia coli
PITINNFRYSDPVNNDTIIMMEPPYCKGLDIYYKAFKITDRIWIVPERYEFGTKPEDFNPPSSLIEGASEYYDPNYLRTDSDKDRFLQTMVKLFNRIKNNVAGEALLDKIINAIPYLGNSYSLLDKFDTNSNSVSFNLLEQDPSGATTKSAMLTNLIIFGPGPVLNKNEVRGIVLRVDNKNYFPCRDGFGSIMQMAFCPEYVPTFDNVIENITSLTIGKSKYFQDPALLLMHELIHVLHGLYGMQVSSHEIIPSKQEIYMQHTYPISAEELFTFGGQDANLISIDIKNDLYEKTLNDYKAIANKLSQVTSCNDPNIDIDSYKQIYQQKYQFDKDSNGQYIVNEDKFQILYNSIMYGFTEIELGKKFNIKTRLSYFSMNHDPVKIPNLLDDTIYNDTEGFNIESKDLKSEYKGQNMRVNTNAFRNVDGSGLVSKLIGLCKKIIPPTNIRENLYNRTASLTDLGGELCIKIKNEDLTFIAEKNSFSEEPFQDEIVSYNTKNKPLNFNYSLDKIIVDYNLQSKITLPNDRTTPVTKGIPYAPEYKSNAASTIEIHNIDDNTIYQYLYAQKSPTTLQRITMTNSVDDALINSTKIYSYFPSVISKVNQGAQGILFLQWVRDIIDDFTNESSQKTTIDKISDVSTIVPYIGPALNIVKQGYEGNFIGALETTGVVLLLEYIPEITLPVIAALSIAESSTQKEKIIKTIDNFLEKRYEKWIEVYKLVKAKWLGTVNTQFQKRSYQMYRSLEYQVDAIKKIIDYEYKIYSGPDKEQIADEINNLKNKLEEKANKAMININIFMRESSRSFLVNQMINEAKKQLLEFDTQSKNILMQYIKANSKFIGITELKKLESKINKVFSTPIPFSYSKNLDCWVDNEEDIDVILKKSTILNLDINNDIISDISGFNSSVITYPDAQLVPGINGKAIHLVNNESSEVIVHKAMDIEYNDMFNNFTVSFWLRVPKVSASHLEQYGTNEYSIISSMKKHSLSIGSGWSVSLKGNNLIWTLKDSAGEVRQITFRDLPDKFNAYLANKWVFITITNDRLSSANLYINGVLMGSAEITGLGAIREDNNITLKLDRCNNNNQYVSIDKFRIFCKALNPKEIEKLYTSYLSITFLRDFWGNPLRYDTEYYLIPVASSSKDVQLKNITDYMYLTNAPSYTNGKLNIYYRRLYNGLKFIIKRYTPNNEIDSFVKSGDFIKLYVSYNNNEHIVGYPKDGNAFNNLDRILEVGYNAPGIPLYKKMEAVKLRDLKTYSVQLKLYDDKNASLGLVGTHNGQIGNDPNRDILIASNAYFNHLKDKILGCDWYFVPTDEGWTND

SEQ ID NO: 11 - DNA, 6816 bp, Escherichia coli
  source 1..6816: mol_type = other DNA
gatctcgatcccgcgaaattaatacgactcactatagggagaccacaacggtttccctctagaaataattttgtttaactttaagaaggagatatacatatgcggggttctcatcatcatcatcatcatggtatggctagcatgactggtggacagcaaatgggtcgggatctgtacgacgatgacgataaggatcgatggggatccgagctcgagccgatcaccatcaacaacttccgttactctgacccggttaacaacgacaccatcatcatgatggaaccgccgtactgcaaaggtctggacatctactacaaagcgttcaaaatcaccgaccgtatctggatcgttccggaacgttacgaattcggtaccaaaccggaagacttcaacccgccgtcttctctgatcgaaggtgcgtctgaatactacgacccgaactacctgcgtaccgactctgacaaagaccgtttcctgcagaccatggttaaactgttcaaccgtatcaaaaacaacgttgcgggtgaagcgctgctggacaaaatcatcaacgcgatcccgtacctgggtaactcttactctctgctggacaaattcgacaccaactctaactctgtttctttcaacctgctggaacaggacccgtctggtgcgaccaccaaatctgcgatgctgaccaacctgatcatcttcggtccgggtccggttctgaacaaaaacgaagttcgtggtatcgttctgcgtgttgacaacaaaaactacttcccgtgccgtgacggtttcggttctatcatgcagatggcgttctgcccggaatacgttccgaccttcgacaacgttatcgaaaacatcacctctctgaccatcggtaaatctaaatacttccaggacccggcgctgctgctgatgcacgaactgatccacgttctgcacggtctgtacggtatgcaggtttcttctcacgaaatcatcccgtctaaacaggaaatctacatgcagcacacctacccgatctctgcggaagaactgttcaccttcggtggtcaggacgcgaacctgatctctatcgacatcaaaaacgacctgtacgaaaaaaccctgaacgactacaaagcgatcgcgaacaaactgtctcaggttacctcttgcaacgacccgaacatcgacatcgactcttacaaacagatctaccagcagaaataccagttcgacaaagactctaacggtcagtacatcgttaacgaagacaaattccagatcctgtacaactctatcatgtacggtttcaccgaaatcgaactgggtaaaaaattcaacatcaaaacccgtctgtcttacttctctatgaaccacgacccggttaaaatcccgaacctgctggacgacaccatctacaacgacaccgaaggtttcaacatcgaatctaaagacctgaaatctgaatacaaaggtcagaacatgcgtgttaacaccaacgcgttccgtaacgttgacggttctggtctggtttctaaactgatcggtctgtgcaaaaaaatcatcccgccgaccaacatccgtgaaaacctgtacaaccgtaccgcgtctctgaccgacctgggtggtgaactgtgcatcaaaatcaaaaacgaagacctgaccttcatcgcggaaaaaaactctttctctgaagaaccgttccaggacgaaatcgtttcttacaacaccaaaaacaaaccgctgaacttcaactactctctggacaaaatcatcgttgactacaacctgcagtctaaaatcaccctgccgaacgaccgtaccaccccggttaccaaaggtatcccgtacgcgccggaatacaaatctaacgcggcgtctaccatcgaaatccacaacatcgacgacaacaccatctaccagtacctgtacgcgcagaaatctccgaccaccctgcagcgtatcaccatgaccaactctgttgacgacgcgctgatcaactctaccaaaatctactcttacttcccgtctgttatctctaaagttaaccagggtgcgcagggtatcctgttcctgcagtgggttcgtgacatcatcgacgacttcaccaacgaatcttctcagaaaaccaccatcgacaaaatctctgacgtttctaccatcgttccgtacatcggtccggcgctgaacatcgttaaacagggttacgaaggtaacttcatcggtgcgctggaaaccaccggtgttgttctgctgctggaatacatcccggaaatcaccctgccggttatcgcggcgctgtctatcgcggaatcttctacccagaaagaaaaaatcatcaaaaccatcgacaacttcctggaaaaacgttacgaaaaatggatcgaagtttacaaactggttaaagcgaaatggctgggtaccgttaacacccagttccagaaacgttcttaccagatgtaccgttctctggaataccaggttgacgcgatcaaaaaaatcatcgactacgaatacaaaatctactctggtccggacaaagaacagatcgcggacgaaatcaacaacctgaaaaacaaactggaagaaaaagcgaacaaagcgatgatcaacatcaacatcttcatgcgtgaatcttctcgttctttcctggttaaccagatgatcaacgaagcgaaaaaacagctgctggaattcgacacccagtctaaaaacatcctgatgcagtacatcaaagcgaactctaaattcatcggtatcaccgaactgaaaaaactggaatctaaaatcaacaaagttttctctaccccgatcccgttctcttactctaaaaacctggactgctgggttgacaacgaagaagacatcgacgttatcctgaaaaaatctaccatcctgaacctggacatcaacaacgacatcatctctgacatctctggtttcaactcttctgttatcacctacccggacgcgcagctggttccgggtatcaacggtaaagcgatccacctggttaacaacgaatcttctgaagttatcgttcacaaagcgatggacatcgaatacaacgacatgttcaacaacttcaccgtttctttctggctgcgtgttccgaaagtttctgcgtctcacctggaacagtacggtaccaacgaatactctatcatctcttctatgaaaaaacactctctgtctatcggttctggttggtctgtttctctgaaaggtaacaacctgatctggaccctgaaagactctgcgggtgaagttcgtcagatcaccttccgtgacctgccggacaaattcaacgcgtacctggcgaacaaatgggttttcatcaccatcaccaacgaccgtctgtcttctgcgaacctgtacatcaacggtgttctgatgggttctgcggaaatcaccggtctgggtgcgatccgtgaagacaacaacatcaccctgaaactggaccgttgcaacaacaacaaccagtacgtttctatcgacaaattccgtatcttctgcaaagcgctgaacccgaaagaaatcgaaaaactgtacacctcttacctgtctatcaccttcctgcgtgacttctggggtaacccgctgcgttacgacaccgaatactacctgatcccggttgcgtcttcttctaaagacgttcagctgaaaaacatcaccgactacatgtacctgaccaacgcgccgtcttacaccaacggtaaactgaacatctactaccgtcgtctgtacaacggtctgaaattcatcatcaaacgttacaccccgaacaacgaaatcgactctttcgttaaatctggtgacttcatcaaactgtacgtttcttacaacaacaacgaacacatcgttggttacccgaaagacggtaacgcgttcaacaacctggaccgtatcctggaagttggttacaacgcgccgggtatcccgctgtacaaaaaaatggaagcggttaaactgcgtgacctgaaaacctactctgttcagctgaaactgtacgacgacaaaaacgcgtctctgggtctggttggtacccacaacggtcagatcggtaacgacccgaaccgtgacatcctgatcgcgtctaacgcgtacttcaaccacctgaaagacaaaatcctgggttgcgactggtacttcgttccgaccgacgaaggttggaccaacgactaaaagcttgatccggctgctaacaaagcccgaaaggaagctgagttggctgctgccaccgctgagcaataactagcataaccccttggggcctctaaacgggtcttgaggggttttttgctgaaaggaggaactatatccggatctggcgtaatagcgaagaggcccgcaccgatcgcccttcccaacagttgcgcagcctgaatggcgaatgggacgcgccctgtagcggcgcattaagcgcggcgggtgtggtggttacgcgcagcgtgaccgctacacttgccagcgccctagcgcccgctcctttcgctttcttcccttcctttctcgccacgttcgccggctttccccgtcaagctctaaatcgggggctccctttagggttccgatttagtgctttacggcacctcgaccccaaaaaacttgattagggtgatggttcacgtagtgggccatcgccctgatagacggtttttcgccctttgacgttggagtccacgttctttaatagtggactcttgttccaaactggaacaacactcaaccctatctcggtctattcttttgatttataagggattttgccgatttcggcctattggttaaaaaatgagctgatttaacaaaaatttaacgcgaattttaacaaaatattaacgcttacaatttaggtggcacttttcggggaaatgtgcgcggaacccctatttgtttatttttctaaatacattcaaatatgtatccgctcatgagacaataaccctgataaatgcttcaataatattgaaaaaggaagagtatgagtattcaacatttccgtgtcgcccttattcccttttttgcggcattttgccttcctgtttttgctcacccagaaacgctggtgaaagtaaaagatgctgaagatcagttgggtgcacgagtgggttacatcgaactggatctcaacagcggtaagatccttgagagttttcgccccgaagaacgttttccaatgatgagcacttttaaagttctgctatgtggcgcggtattatcccgtattgacgccgggcaagagcaactcggtcgccgcatacactattctcagaatgacttggttgagtactcaccagtcacagaaaagcatcttacggatggcatgacagtaagagaattatgcagtgctgccataaccatgagtgataacactgcggccaacttacttctgacaacgatcggaggaccgaaggagctaaccgcttttttgcacaacatgggggatcatgtaactcgccttgatcgttgggaaccggagctgaatgaagccataccaaacgacgagcgtgacaccacgatgcctgtagcaatggcaacaacgttgcgcaaactattaactggcgaactacttactctagcttcccggcaacaattaatagactggatggaggcggataaagttgcaggaccacttctgcgctcggcccttccggctggctggtttattgctgataaatctggagccggtgagcgtgggtctcgcggtatcattgcagcactggggccagatggtaagccctcccgtatcgtagttatctacacgacggggagtcaggcaactatggatgaacgaaatagacagatcgctgagataggtgcctcactgattaagcattggtaactgtcagaccaagtttactcatatatactttagattgatttaaaacttcatttttaatttaaaaggatctaggtgaagatcctttttgataatctcatgaccaaaatcccttaacgtgagttttcgttccactgagcgtcagaccccgtagaaaagatcaaaggatcttcttgagatcctttttttctgcgcgtaatctgctgcttgcaaacaaaaaaaccaccgctaccagcggtggtttgtttgccggatcaagagctaccaactctttttccgaaggtaactggcttcagcagagcgcagataccaaatactgttcttctagtgtagccgtagttaggccaccacttcaagaactctgtagcaccgcctacatacctcgctctgctaatcctgttaccagtggctgctgccagtggcgataagtcgtgtcttaccgggttggactcaagacgatagttaccggataaggcgcagcggtcgggctgaacggggggttcgtgcacacagcccagcttggagcgaacgacctacaccgaactgagatacctacagcgtgagctatgagaaagcgccacgcttcccgaagggagaaaggcggacaggtatccggtaagcggcagggtcggaacaggagagcgcacgagggagcttccagggggaaacgcctggtatctttatagtcctgtcgggtttcgccacctctgacttgagcgtcgatttttgtgatgctcgtcaggggggcggagcctatggaaaaacgccagcaacgcggcctttttacggttcctggccttttgctggccttttgctcacatgttctttcctgcgttatcccctgattctgtggataaccgtattaccgcctttgagtgagctgataccgctcgccgcagccgaacgaccgagcgcagcgagtcagtgagcgaggaagcggaagagcgcccaatacgcaaaccgcctctccccgcgcgttggccgattcattaatgcag

SEQ ID NO: 12 - protein, 1314 aa, Escherichia coli
PITINNFRYSDPVNNDTIIMMEPPYCKGLDIYYKAFKITDRIWIVPERYEFGTKPEDFNPPSSLIEGASEYYDPNYLRTDCDKDRFLQTMVKLFNRIKNNVAGEALLDKIINAIPYLGNCYSLLDKFDTNSNSVSFNLLEQDPCGATTKSAMLTNLIIFGPGPVLNKNEVRGIVLRVDNKNYFPCRDGFGSIMQMAFCPEYVPTFDNVIENITSLTIGKSKYFQDPALLLMHELIHVLHGLYGMQVSCHEIIPSKQEIYMQHTYPISAEELFTFGGQDANLISIDIKNDLYEKTLNDYKAIANKLSQVTSCNDPNIDIDSYKQIYQQKYQFDKDCNGQYIVNEDKFQILYNSIMYGFTEIELGKKFNIKTRLSYFSMNHDPVKIPNLLDDTIYNDTEGFNIESKDLKSEYKGQNMRVNTNAFRNVDGCGLVSKLIGLCKKIIPPTNIRENLYNRTASLTDLGGELCIKIKNEDLTFIAEKNSFSEEPFQDEIVSYNTKNKPLNFNYSLDKIIVDYNLQSKITLPNDRTTPVTKGIPYAPEYKSNAASTIEIHNIDDNTIYQYLYAQKSPTTLQRITMTNSVDDALINSTKIYSYFPSVICKVNQGAQGILFLQWVRDIIDDFTNESSQKTTIDKISDVSTIVPYIGPALNIVKQGYEGNFIGALETTGVVLLLEYIPEITLPVIAALSIAESSTQKEKIIKTIDNFLEKRYEKWIEVYKLVKAKWLGTVNTQFQKRSYQMYRSLEYQVDAIKKIIDYEYKIYSGPDKEQIADEINNLKNKLEEKANKAMININIFMRESSRSFLVNQMINEAKKQLLEFDTQSKNILMQYIKANSKFIGITELKKLESKINKVFSTPIPFSYSKNLDCWVDNEEDIDVILKKSTILNLDINNDIISDISGFNSSVITYPDAQLVPGINGKAIHLVNNESSEVIVHKAMDIEYNDMFNNFTVSFWLRVPKVSACHLEQYGTNEYSIISSMKKHSLSIGSGWSVSLKGNNLIWTLKDSAGEVRQITFRDLPDKFNAYLANKWVFITITNDRLCSANLYINGVLMGSAEITGLGAIREDNNITLKLDRCNNNNQYVSIDKFRIFCKALNPKEIEKLYTSYLSITFLRDFWGNPLRYDTEYYLIPVASSSKDVQLKNITDYMYLTNAPCYTNGKLNIYYRRLYNGLKFIIKRYTPNNEIDCFVKSGDFIKLYVSYNNNEHIVGYPKDGNAFNNLDRILRVGYNAPGIPLYKKMEAVKLRDLKTYSVQLKLYDDKNASLGLVGTHNGQIGNDPNRDILIASNWYFNHLKDKILGCDWYFVPTDEGWTND

SEQ ID NO: 13 - DNA, 6816 bp, Escherichia coli
  source 1..6816: mol_type = other DNA
gatctcgatcccgcgaaattaatacgactcactatagggagaccacaacggtttccctctagaaataattttgtttaactttaagaaggagatatacatatgcggggttctcatcatcatcatcatcatggtatggctagcatgactggtggacagcaaatgggtcgggatctgtacgacgatgacgataaggatcgatggggatccgagctcgagccgatcaccatcaacaacttccgttactctgacccggttaacaacgacaccatcatcatgatggaaccgccgtactgcaaaggtctggacatctactacaaagcgttcaaaatcaccgaccgtatctggatcgttccggaacgttacgaattcggtaccaaaccggaagacttcaacccgccgtcttctctgatcgaaggtgcgtctgaatactacgacccgaactacctgcgtaccgactgcgacaaagaccgtttcctgcagaccatggttaaactgttcaaccgtatcaaaaacaacgttgcgggtgaagcgctgctggacaaaatcatcaacgcgatcccgtacctgggtaactgctactctctgctggacaaattcgacaccaactctaactctgtttctttcaacctgctggaacaggacccgtgcggtgcgaccaccaaatctgcgatgctgaccaacctgatcatcttcggtccgggtccggttctgaacaaaaacgaagttcgtggtatcgttctgcgtgttgacaacaaaaactacttcccgtgccgtgacggtttcggttctatcatgcagatggcgttctgcccggaatacgttccgaccttcgacaacgttatcgaaaacatcacctctctgaccatcggtaaatctaaatacttccaggacccggcgctgctgctgatgcacgaactgatccacgttctgcacggtctgtacggtatgcaggtttcttgccacgaaatcatcccgtctaaacaggaaatctacatgcagcacacctacccgatctctgcggaagaactgttcaccttcggtggtcaggacgcgaacctgatctctatcgacatcaaaaacgacctgtacgaaaaaaccctgaacgactacaaagcgatcgcgaacaaactgtctcaggttacctcttgcaacgacccgaacatcgacatcgactcttacaaacagatctaccagcagaaataccagttcgacaaagactgcaacggtcagtacatcgttaacgaagacaaattccagatcctgtacaactctatcatgtacggtttcaccgaaatcgaactgggtaaaaaattcaacatcaaaacccgtctgtcttacttctctatgaaccacgacccggttaaaatcccgaacctgctggacgacaccatctacaacgacaccgaaggtttcaacatcgaatctaaagacctgaaatctgaatacaaaggtcagaacatgcgtgttaacaccaacgcgttccgtaacgttgacggttgcggtctggtttctaaactgatcggtctgtgcaaaaaaatcatcccgccgaccaacatccgtgaaaacctgtacaaccgtaccgcgtctctgaccgacctgggtggtgaactgtgcatcaaaatcaaaaacgaagacctgaccttcatcgcggaaaaaaactctttctctgaagaaccgttccaggacgaaatcgtttcttacaacaccaaaaacaaaccgctgaacttcaactactctctggacaaaatcatcgttgactacaacctgcagtctaaaatcaccctgccgaacgaccgtaccaccccggttaccaaaggtatcccgtacgcgccggaatacaaatctaacgcggcgtctaccatcgaaatccacaacatcgacgacaacaccatctaccagtacctgtacgcgcagaaatctccgaccaccctgcagcgtatcaccatgaccaactctgttgacgacgcgctgatcaactctaccaaaatctactcttacttcccgtctgttatctgcaaagttaaccagggtgcgcagggtatcctgttcctgcagtgggttcgtgacatcatcgacgacttcaccaacgaatcttctcagaaaaccaccatcgacaaaatctctgacgtttctaccatcgttccgtacatcggtccggcgctgaacatcgttaaacagggttacgaaggtaacttcatcggtgcgctggaaaccaccggtgttgttctgctgctggaatacatcccggaaatcaccctgccggttatcgcggcgctgtctatcgcggaatcttctacccagaaagaaaaaatcatcaaaaccatcgacaacttcctggaaaaacgttacgaaaaatggatcgaagtttacaaactggttaaagcgaaatggctgggtaccgttaacacccagttccagaaacgttcttaccagatgtaccgttctctggaataccaggttgacgcgatcaaaaaaatcatcgactacgaatacaaaatctactctggtccggacaaagaacagatcgcggacgaaatcaacaacctgaaaaacaaactggaagaaaaagcgaacaaagcgatgatcaacatcaacatcttcatgcgtgaatcttctcgttctttcctggttaaccagatgatcaacgaagcgaaaaaacagctgctggaattcgacacccagtctaaaaacatcctgatgcagtacatcaaagcgaactctaaattcatcggtatcaccgaactgaaaaaactggaatctaaaatcaacaaagttttctctaccccgatcccgttctcttactctaaaaacctggactgctgggttgacaacgaagaagacatcgacgttatcctgaaaaaatctaccatcctgaacctggacatcaacaacgacatcatctctgacatctctggtttcaactcttctgttatcacctacccggacgcgcagctggttccgggtatcaacggtaaagcgatccacctggttaacaacgaatcttctgaagttatcgttcacaaagcgatggacatcgaatacaacgacatgttcaacaacttcaccgtttctttctggctgcgtgttccgaaagtttctgcgtgccacctggaacagtacggtaccaacgaatactctatcatctcttctatgaaaaaacactctctgtctatcggttctggttggtctgtttctctgaaaggtaacaacctgatctggaccctgaaagactctgcgggtgaagttcgtcagatcaccttccgtgacctgccggacaaattcaacgcgtacctggcgaacaaatgggttttcatcaccatcaccaacgaccgtctgtgctctgcgaacctgtacatcaacggtgttctgatgggttctgcggaaatcaccggtctgggtgcgatccgtgaagacaacaacatcaccctgaaactggaccgttgcaacaacaacaaccagtacgtttctatcgacaaattccgtatcttctgcaaagcgctgaacccgaaagaaatcgaaaaactgtacacctcttacctgtctatcaccttcctgcgtgacttctggggtaacccgctgcgttacgacaccgaatactacctgatcccggttgcgtcttcttctaaagacgttcagctgaaaaacatcaccgactacatgtacctgaccaacgcgccgtgctacaccaacggtaaactgaacatctactaccgtcgtctgtacaacggtctgaaattcatcatcaaacgttacaccccgaacaacgaaatcgactgcttcgttaaatctggtgacttcatcaaactgtacgtttcttacaacaacaacgaacacatcgttggttacccgaaagacggtaacgcgttcaacaacctggaccgtatcctgcgtgttggttacaacgcgccgggtatcccgctgtacaaaaaaatggaagcggttaaactgcgtgacctgaaaacctactctgttcagctgaaactgtacgacgacaaaaacgcgtctctgggtctggttggtacccacaacggtcagatcggtaacgacccgaaccgtgacatcctgatcgcgtctaactggtacttcaaccacctgaaagacaaaatcctgggttgcgactggtacttcgttccgaccgacgaaggttggaccaacgactaaaagcttgatccggctgctaacaaagcccgaaaggaagctgagttggctgctgccaccgctgagcaataactagcataaccccttggggcctctaaacgggtcttgaggggttttttgctgaaaggaggaactatatccggatctggcgtaatagcgaagaggcccgcaccgatcgcccttcccaacagttgcgcagcctgaatggcgaatgggacgcgccctgtagcggcgcattaagcgcggcgggtgtggtggttacgcgcagcgtgaccgctacacttgccagcgccctagcgcccgctcctttcgctttcttcccttcctttctcgccacgttcgccggctttccccgtcaagctctaaatcgggggctccctttagggttccgatttagtgctttacggcacctcgaccccaaaaaacttgattagggtgatggttcacgtagtgggccatcgccctgatagacggtttttcgccctttgacgttggagtccacgttctttaatagtggactcttgttccaaactggaacaacactcaaccctatctcggtctattcttttgatttataagggattttgccgatttcggcctattggttaaaaaatgagctgatttaacaaaaatttaacgcgaattttaacaaaatattaacgcttacaatttaggtggcacttttcggggaaatgtgcgcggaacccctatttgtttatttttctaaatacattcaaatatgtatccgctcatgagacaataaccctgataaatgcttcaataatattgaaaaaggaagagtatgagtattcaacatttccgtgtcgcccttattcccttttttgcggcattttgccttcctgtttttgctcacccagaaacgctggtgaaagtaaaagatgctgaagatcagttgggtgcacgagtgggttacatcgaactggatctcaacagcggtaagatccttgagagttttcgccccgaagaacgttttccaatgatgagcacttttaaagttctgctatgtggcgcggtattatcccgtattgacgccgggcaagagcaactcggtcgccgcatacactattctcagaatgacttggttgagtactcaccagtcacagaaaagcatcttacggatggcatgacagtaagagaattatgcagtgctgccataaccatgagtgataacactgcggccaacttacttctgacaacgatcggaggaccgaaggagctaaccgcttttttgcacaacatgggggatcatgtaactcgccttgatcgttgggaaccggagctgaatgaagccataccaaacgacgagcgtgacaccacgatgcctgtagcaatggcaacaacgttgcgcaaactattaactggcgaactacttactctagcttcccggcaacaattaatagactggatggaggcggataaagttgcaggaccacttctgcgctcggcccttccggctggctggtttattgctgataaatctggagccggtgagcgtgggtctcgcggtatcattgcagcactggggccagatggtaagccctcccgtatcgtagttatctacacgacggggagtcaggcaactatggatgaacgaaatagacagatcgctgagataggtgcctcactgattaagcattggtaactgtcagaccaagtttactcatatatactttagattgatttaaaacttcatttttaatttaaaaggatctaggtgaagatcctttttgataatctcatgaccaaaatcccttaacgtgagttttcgttccactgagcgtcagaccccgtagaaaagatcaaaggatcttcttgagatcctttttttctgcgcgtaatctgctgcttgcaaacaaaaaaaccaccgctaccagcggtggtttgtttgccggatcaagagctaccaactctttttccgaaggtaactggcttcagcagagcgcagataccaaatactgttcttctagtgtagccgtagttaggccaccacttcaagaactctgtagcaccgcctacatacctcgctctgctaatcctgttaccagtggctgctgccagtggcgataagtcgtgtcttaccgggttggactcaagacgatagttaccggataaggcgcagcggtcgggctgaacggggggttcgtgcacacagcccagcttggagcgaacgacctacaccgaactgagatacctacagcgtgagctatgagaaagcgccacgcttcccgaagggagaaaggcggacaggtatccggtaagcggcagggtcggaacaggagagcgcacgagggagcttccagggggaaacgcctggtatctttatagtcctgtcgggtttcgccacctctgacttgagcgtcgatttttgtgatgctcgtcaggggggcggagcctatggaaaaacgccagcaacgcggcctttttacggttcctggccttttgctggccttttgctcacatgttctttcctgcgttatcccctgattctgtggataaccgtattaccgcctttgagtgagctgataccgctcgccgcagccgaacgaccgagcgcagcgagtcagtgagcgaggaagcggaagagcgcccaatacgcaaaccgcctctccccgcgcgttggccgattcattaatgcag

SEQ ID NO: 14 - protein, 1314 aa, Escherichia coli
PITINNFRYSDPVNNDTIIMMEPPYCKGLDIYYKAFKITDRIWIVPERYEFGTKPEDFNPPSSLIEGASEYYDPNYLRTDCDKDRFLQTMVKLFNRIKNNVAGEALLDKIINAIPYLGNCYSLLDKFDTNSNSVSFNLLEQDPCGATTKSAMLTNLIIFGPGPVLNKNEVRGIVLRVDNKNYFPCRDGFGSIMQMAFCPEYVPTFDNVIENITSLTIGKSKYFQDPALLLMHELIHVLHGLYGMQVSCHEIIPSKQEIYMQHTYPISAEELFTFGGQDANLISIDIKNDLYEKTLNDYKAIANKLSQVTSCNDPNIDIDSYKQIYQQKYQFDKDCNGQYIVNEDKFQILYNSIMYGFTEIELGKKFNIKTRLSYFSMNHDPVKIPNLLDDTIYNDTEGFNIESKDLKSEYKGQNMRVNTNAFRNVDGCGLVSKLIGLCKKIIPPTNIRENLYNRTASLTDLGGELCIKIKNEDLTFIAEKNSFSEEPFQDEIVSYNTKNKPLNFNYSLDKIIVDYNLQSKITLPNDRTTPVTKGIPYAPEYKSNAASTIEIHNIDDNTIYQYLYAQKSPTTLQRITMTNSVDDALINSTKIYSYFPSVISKVNQGAQGILFLQWVRDIIDDFTNESSQKTTIDKISDVSTIVPYIGPALNIVKQGYEGNFIGALETTGVVLLLEYIPEITLPVIAALSIAESSTQKEKIIKTIDNFLEKRYEKWIEVYKLVKAKWLGTVNTQFQKRSYQMYRSLEYQVDAIKKIIDYEYKIYSGPDKEQIADEINNLKNKLEEKANKAMININIFMRESSRSFLVNQMINEAKKQLLEFDTQSKNILMQYIKANSKFIGITELKKLESKINKVFSTPIPFSYSKNLDCWVDNEEDIDVILKKSTILNLDINNDIISDISGFNSSVITYPDAQLVPGINGKAIHLVNNESSEVIVHKAMDIEYNDMFNNFTVSFWLRVPKVSACHLEQYGTNEYSIISSMKKHSLSIGSGWSVSLKGNNLIWTLKDSAGEVRQITFRDLPDKFNAYLANKWVFITITNDRLCSANLYINGVLMGSAEITGLGAIREDNNITLKLDRCNNNNQYVSIDKFRIFCKALNPKEIEKLYTSYLSITFLRDFWGNPLRYDTEYYLIPVASSSKDVQLKNITDYMYLTNAPCYTNGKLNIYYRRLYNGLKFIIKRYTPNNEIDCFVKSGDFIKLYVSYNNNEHIVGYPKDGNAFNNLDRILRVGYNAPGIPLYKKMEAVKLRDLKTYSVQLKLYDDKNASLGLVGTHNGQIGNDPNRDILIASNWYFNHLKDKILGCDWYFVPTDEGWTND

SEQ ID NO: 15 - DNA, 6816 bp, Escherichia coli
  source 1..6816: mol_type = other DNA
gatctcgatcccgcgaaattaatacgactcactatagggagaccacaacggtttccctctagaaataattttgtttaactttaagaaggagatatacatatgcggggttctcatcatcatcatcatcatggtatggctagcatgactggtggacagcaaatgggtcgggatctgtacgacgatgacgataaggatcgatggggatccgagctcgagccgatcaccatcaacaacttccgttactctgacccggttaacaacgacaccatcatcatgatggaaccgccgtactgcaaaggtctggacatctactacaaagcgttcaaaatcaccgaccgtatctggatcgttccggaacgttacgaattcggtaccaaaccggaagacttcaacccgccgtcttctctgatcgaaggtgcgtctgaatactacgacccgaactacctgcgtaccgactgcgacaaagaccgtttcctgcagaccatggttaaactgttcaaccgtatcaaaaacaacgttgcgggtgaagcgctgctggacaaaatcatcaacgcgatcccgtacctgggtaactgctactctctgctggacaaattcgacaccaactctaactctgtttctttcaacctgctggaacaggacccgtgcggtgcgaccaccaaatctgcgatgctgaccaacctgatcatcttcggtccgggtccggttctgaacaaaaacgaagttcgtggtatcgttctgcgtgttgacaacaaaaactacttcccgtgccgtgacggtttcggttctatcatgcagatggcgttctgcccggaatacgttccgaccttcgacaacgttatcgaaaacatcacctctctgaccatcggtaaatctaaatacttccaggacccggcgctgctgctgatgcacgaactgatccacgttctgcacggtctgtacggtatgcaggtttcttgccacgaaatcatcccgtctaaacaggaaatctacatgcagcacacctacccgatctctgcggaagaactgttcaccttcggtggtcaggacgcgaacctgatctctatcgacatcaaaaacgacctgtacgaaaaaaccctgaacgactacaaagcgatcgcgaacaaactgtctcaggttacctcttgcaacgacccgaacatcgacatcgactcttacaaacagatctaccagcagaaataccagttcgacaaagactgcaacggtcagtacatcgttaacgaagacaaattccagatcctgtacaactctatcatgtacggtttcaccgaaatcgaactgggtaaaaaattcaacatcaaaacccgtctgtcttacttctctatgaaccacgacccggttaaaatcccgaacctgctggacgacaccatctacaacgacaccgaaggtttcaacatcgaatctaaagacctgaaatctgaatacaaaggtcagaacatgcgtgttaacaccaacgcgttccgtaacgttgacggttgcggtctggtttctaaactgatcggtctgtgcaaaaaaatcatcccgccgaccaacatccgtgaaaacctgtacaaccgtaccgcgtctctgaccgacctgggtggtgaactgtgcatcaaaatcaaaaacgaagacctgaccttcatcgcggaaaaaaactctttctctgaagaaccgttccaggacgaaatcgtttcttacaacaccaaaaacaaaccgctgaacttcaactactctctggacaaaatcatcgttgactacaacctgcagtctaaaatcaccctgccgaacgaccgtaccaccccggttaccaaaggtatcccgtacgcgccggaatacaaatctaacgcggcgtctaccatcgaaatccacaacatcgacgacaacaccatctaccagtacctgtacgcgcagaaatctccgaccaccctgcagcgtatcaccatgaccaactctgttgacgacgcgctgatcaactctaccaaaatctactcttacttcccgtctgttatctctaaagttaaccagggtgcgcagggtatcctgttcctgcagtgggttcgtgacatcatcgacgacttcaccaacgaatcttctcagaaaaccaccatcgacaaaatctctgacgtttctaccatcgttccgtacatcggtccggcgctgaacatcgttaaacagggttacgaaggtaacttcatcggtgcgctggaaaccaccggtgttgttctgctgctggaatacatcccggaaatcaccctgccggttatcgcggcgctgtctatcgcggaatcttctacccagaaagaaaaaatcatcaaaaccatcgacaacttcctggaaaaacgttacgaaaaatggatcgaagtttacaaactggttaaagcgaaatggctgggtaccgttaacacccagttccagaaacgttcttaccagatgtaccgttctctggaataccaggttgacgcgatcaaaaaaatcatcgactacgaatacaaaatctactctggtccggacaaagaacagatcgcggacgaaatcaacaacctgaaaaacaaactggaagaaaaagcgaacaaagcgatgatcaacatcaacatcttcatgcgtgaatcttctcgttctttcctggttaaccagatgatcaacgaagcgaaaaaacagctgctggaattcgacacccagtctaaaaacatcctgatgcagtacatcaaagcgaactctaaattcatcggtatcaccgaactgaaaaaactggaatctaaaatcaacaaagttttctctaccccgatcccgttctcttactctaaaaacctggactgctgggttgacaacgaagaagacatcgacgttatcctgaaaaaatctaccatcctgaacctggacatcaacaacgacatcatctctgacatctctggtttcaactcttctgttatcacctacccggacgcgcagctggttccgggtatcaacggtaaagcgatccacctggttaacaacgaatcttctgaagttatcgttcacaaagcgatggacatcgaatacaacgacatgttcaacaacttcaccgtttctttctggctgcgtgttccgaaagtttctgcgtgccacctggaacagtacggtaccaacgaatactctatcatctcttctatgaaaaaacactctctgtctatcggttctggttggtctgtttctctgaaaggtaacaacctgatctggaccctgaaagactctgcgggtgaagttcgtcagatcaccttccgtgacctgccggacaaattcaacgcgtacctggcgaacaaatgggttttcatcaccatcaccaacgaccgtctgtgctctgcgaacctgtacatcaacggtgttctgatgggttctgcggaaatcaccggtctgggtgcgatccgtgaagacaacaacatcaccctgaaactggaccgttgcaacaacaacaaccagtacgtttctatcgacaaattccgtatcttctgcaaagcgctgaacccgaaagaaatcgaaaaactgtacacctcttacctgtctatcaccttcctgcgtgacttctggggtaacccgctgcgttacgacaccgaatactacctgatcccggttgcgtcttcttctaaagacgttcagctgaaaaacatcaccgactacatgtacctgaccaacgcgccgtgctacaccaacggtaaactgaacatctactaccgtcgtctgtacaacggtctgaaattcatcatcaaacgttacaccccgaacaacgaaatcgactgcttcgttaaatctggtgacttcatcaaactgtacgtttcttacaacaacaacgaacacatcgttggttacccgaaagacggtaacgcgttcaacaacctggaccgtatcctgcgtgttggttacaacgcgccgggtatcccgctgtacaaaaaaatggaagcggttaaactgcgtgacctgaaaacctactctgttcagctgaaactgtacgacgacaaaaacgcgtctctgggtctggttggtacccacaacggtcagatcggtaacgacccgaaccgtgacatcctgatcgcgtctaactggtacttcaaccacctgaaagacaaaatcctgggttgcgactggtacttcgttccgaccgacgaaggttggaccaacgactaaaagcttgatccggctgctaacaaagcccgaaaggaagctgagttggctgctgccaccgctgagcaataactagcataaccccttggggcctctaaacgggtcttgaggggttttttgctgaaaggaggaactatatccggatctggcgtaatagcgaagaggcccgcaccgatcgcccttcccaacagttgcgcagcctgaatggcgaatgggacgcgccctgtagcggcgcattaagcgcggcgggtgtggtggttacgcgcagcgtgaccgctacacttgccagcgccctagcgcccgctcctttcgctttcttcccttcctttctcgccacgttcgccggctttccccgtcaagctctaaatcgggggctccctttagggttccgatttagtgctttacggcacctcgaccccaaaaaacttgattagggtgatggttcacgtagtgggccatcgccctgatagacggtttttcgccctttgacgttggagtccacgttctttaatagtggactcttgttccaaactggaacaacactcaaccctatctcggtctattcttttgatttataagggattttgccgatttcggcctattggttaaaaaatgagctgatttaacaaaaatttaacgcgaattttaacaaaatattaacgcttacaatttaggtggcacttttcggggaaatgtgcgcggaacccctatttgtttatttttctaaatacattcaaatatgtatccgctcatgagacaataaccctgataaatgcttcaataatattgaaaaaggaagagtatgagtattcaacatttccgtgtcgcccttattcccttttttgcggcattttgccttcctgtttttgctcacccagaaacgctggtgaaagtaaaagatgctgaagatcagttgggtgcacgagtgggttacatcgaactggatctcaacagcggtaagatccttgagagttttcgccccgaagaacgttttccaatgatgagcacttttaaagttctgctatgtggcgcggtattatcccgtattgacgccgggcaagagcaactcggtcgccgcatacactattctcagaatgacttggttgagtactcaccagtcacagaaaagcatcttacggatggcatgacagtaagagaattatgcagtgctgccataaccatgagtgataacactgcggccaacttacttctgacaacgatcggaggaccgaaggagctaaccgcttttttgcacaacatgggggatcatgtaactcgccttgatcgttgggaaccggagctgaatgaagccataccaaacgacgagcgtgacaccacgatgcctgtagcaatggcaacaacgttgcgcaaactattaactggcgaactacttactctagcttcccggcaacaattaatagactggatggaggcggataaagttgcaggaccacttctgcgctcggcccttccggctggctggtttattgctgataaatctggagccggtgagcgtgggtctcgcggtatcattgcagcactggggccagatggtaagccctcccgtatcgtagttatctacacgacggggagtcaggcaactatggatgaacgaaatagacagatcgctgagataggtgcctcactgattaagcattggtaactgtcagaccaagtttactcatatatactttagattgatttaaaacttcatttttaatttaaaaggatctaggtgaagatcctttttgataatctcatgaccaaaatcccttaacgtgagttttcgttccactgagcgtcagaccccgtagaaaagatcaaaggatcttcttgagatcctttttttctgcgcgtaatctgctgcttgcaaacaaaaaaaccaccgctaccagcggtggtttgtttgccggatcaagagctaccaactctttttccgaaggtaactggcttcagcagagcgcagataccaaatactgttcttctagtgtagccgtagttaggccaccacttcaagaactctgtagcaccgcctacatacctcgctctgctaatcctgttaccagtggctgctgccagtggcgataagtcgtgtcttaccgggttggactcaagacgatagttaccggataaggcgcagcggtcgggctgaacggggggttcgtgcacacagcccagcttggagcgaacgacctacaccgaactgagatacctacagcgtgagctatgagaaagcgccacgcttcccgaagggagaaaggcggacaggtatccggtaagcggcagggtcggaacaggagagcgcacgagggagcttccagggggaaacgcctggtatctttatagtcctgtcgggtttcgccacctctgacttgagcgtcgatttttgtgatgctcgtcaggggggcggagcctatggaaaaacgccagcaacgcggcctttttacggttcctggccttttgctggccttttgctcacatgttctttcctgcgttatcccctgattctgtggataaccgtattaccgcctttgagtgagctgataccgctcgccgcagccgaacgaccgagcgcagcgagtcagtgagcgaggaagcggaagagcgcccaatacgcaaaccgcctctccccgcgcgttggccgattcattaatgcag

SEQ ID NO: 16 - protein, 1314 aa, Escherichia coli
PITINNFRYSDPVNNDTIIMMEPPYCKGLDIYYKAFKITDRIWIVPERYEFGTKPEDFNPPSSLIEGASEYYDPNYLRTDSDKDRFLQTMVKLFNRIKNNVAGEALLDKIINAIPYLGNSYSLLDKFDTNSNSVSFNLLEQDPSGATTKSAMLTNLIIFGPGPVLNKNEVRGIVLRVDNKNYFPCRDGFGSIMQMAFCPEYVPTFDNVIENITSLTIGKSKYFQDPALLLMHELIHVLHGLYGMQVSSHEIIPSKQEIYMQHTYPISAEELFTFGGQDANLISIDIKNDLYEKTLNDYKAIANKLSQVTSCNDPNIDIDSYKQIYQQKYQFDKDSNGQYIVNEDKFQILYNSIMYGFTEIELGKKFNIKTRLSYFSMNHDPVKIPNLLDDTIYNDTEGFNIESKDLKSEYKGQNMRVNTNAFRNVDGSGLVSKLIGLCKKIIPPTNIRENLYNRTASLTDLGGELCIKIKNEDLTFIAEKNSFSEEPFQDEIVSYNTKNKPLNFNYSLDKIIVDYNLQSKITLPNDRTTPVTKGIPYAPEYKSNAASTIEIHNIDDNTIYQYLYAQKSPTTLQRITMTNSVDDALINSTKIYSYFPSVICKVNQGAQGILFLQWVRDIIDDFTNESSQKTTIDKISDVSTIVPYIGPALNIVKQGYEGNFIGALETTGVVLLLEYIPEITLPVIAALSIAESSTQKEKIIKTIDNFLEKRYEKWIEVYKLVKAKWLGTVNTQFQKRSYQMYRSLEYQVDAIKKIIDYEYKIYSGPDKEQIADEINNLKNKLEEKANKAMININIFMRESSRSFLVNQMINEAKKQLLEFDTQSKNILMQYIKANSKFIGITELKKLESKINKVFSTPIPFSYSKNLDCWVDNEEDIDVILKKSTILNLDINNDIISDISGFNSSVITYPDAQLVPGINGKAIHLVNNESSEVIVHKAMDIEYNDMFNNFTVSFWLRVPKVSACHLEQYGTNEYSIISSMKKHSLSIGSGWSVSLKGNNLIWTLKDSAGEVRQITFRDLPDKFNAYLANKWVFITITNDRLCSANLYINGVLMGSAEITGLGAIREDNNITLKLDRCNNNNQYVSIDKFRIFCKALNPKEIEKLYTSYLSITFLRDFWGNPLRYDTEYYLIPVASSSKDVQLKNITDYMYLTNAPCYTNGKLNIYYRRLYNGLKFIIKRYTPNNEIDCFVKSGDFIKLYVSYNNNEHIVGYPKDGNAFNNLDRILRVGYNAPGIPLYKKMEAVKLRDLKTYSVQLKLYDDKNASLGLVGTHNGQIGNDPNRDILIASNWYFNHLKDKILGCDWYFVPTDEGWTND

SEQ ID NO: 17 - DNA, 6816 bp, Escherichia coli
  source 1..6816: mol_type = other DNA
gatctcgatcccgcgaaattaatacgactcactatagggagaccacaacggtttccctctagaaataattttgtttaactttaagaaggagatatacatatgcggggttctcatcatcatcatcatcatggtatggctagcatgactggtggacagcaaatgggtcgggatctgtacgacgatgacgataaggatcgatggggatccgagctcgagccgatcaccatcaacaacttccgttactctgacccggttaacaacgacaccatcatcatgatggaaccgccgtactgcaaaggtctggacatctactacaaagcgttcaaaatcaccgaccgtatctggatcgttccggaacgttacgaattcggtaccaaaccggaagacttcaacccgccgtcttctctgatcgaaggtgcgtctgaatactacgacccgaactacctgcgtaccgactctgacaaagaccgtttcctgcagaccatggttaaactgttcaaccgtatcaaaaacaacgttgcgggtgaagcgctgctggacaaaatcatcaacgcgatcccgtacctgggtaactcttactctctgctggacaaattcgacaccaactctaactctgtttctttcaacctgctggaacaggacccgtctggtgcgaccaccaaatctgcgatgctgaccaacctgatcatcttcggtccgggtccggttctgaacaaaaacgaagttcgtggtatcgttctgcgtgttgacaacaaaaactacttcccgtgccgtgacggtttcggttctatcatgcagatggcgttctgcccggaatacgttccgaccttcgacaacgttatcgaaaacatcacctctctgaccatcggtaaatctaaatacttccaggacccggcgctgctgctgatgcacgaactgatccacgttctgcacggtctgtacggtatgcaggtttcttctcacgaaatcatcccgtctaaacaggaaatctacatgcagcacacctacccgatctctgcggaagaactgttcaccttcggtggtcaggacgcgaacctgatctctatcgacatcaaaaacgacctgtacgaaaaaaccctgaacgactacaaagcgatcgcgaacaaactgtctcaggttacctcttgcaacgacccgaacatcgacatcgactcttacaaacagatctaccagcagaaataccagttcgacaaagactctaacggtcagtacatcgttaacgaagacaaattccagatcctgtacaactctatcatgtacggtttcaccgaaatcgaactgggtaaaaaattcaacatcaaaacccgtctgtcttacttctctatgaaccacgacccggttaaaatcccgaacctgctggacgacaccatctacaacgacaccgaaggtttcaacatcgaatctaaagacctgaaatctgaatacaaaggtcagaacatgcgtgttaacaccaacgcgttccgtaacgttgacggttctggtctggtttctaaactgatcggtctgtgcaaaaaaatcatcccgccgaccaacatccgtgaaaacctgtacaaccgtaccgcgtctctgaccgacctgggtggtgaactgtgcatcaaaatcaaaaacgaagacctgaccttcatcgcggaaaaaaactctttctctgaagaaccgttccaggacgaaatcgtttcttacaacaccaaaaacaaaccgctgaacttcaactactctctggacaaaatcatcgttgactacaacctgcagtctaaaatcaccctgccgaacgaccgtaccaccccggttaccaaaggtatcccgtacgcgccggaatacaaatctaacgcggcgtctaccatcgaaatccacaacatcgacgacaacaccatctaccagtacctgtacgcgcagaaatctccgaccaccctgcagcgtatcaccatgaccaactctgttgacgacgcgctgatcaactctaccaaaatctactcttacttcccgtctgttatctgcaaagttaaccagggtgcgcagggtatcctgttcctgcagtgggttcgtgacatcatcgacgacttcaccaacgaatcttctcagaaaaccaccatcgacaaaatctctgacgtttctaccatcgttccgtacatcggtccggcgctgaacatcgttaaacagggttacgaaggtaacttcatcggtgcgctggaaaccaccggtgttgttctgctgctggaatacatcccggaaatcaccctgccggttatcgcggcgctgtctatcgcggaatcttctacccagaaagaaaaaatcatcaaaaccatcgacaacttcctggaaaaacgttacgaaaaatggatcgaagtttacaaactggttaaagcgaaatggctgggtaccgttaacacccagttccagaaacgttcttaccagatgtaccgttctctggaataccaggttgacgcgatcaaaaaaatcatcgactacgaatacaaaatctactctggtccggacaaagaacagatcgcggacgaaatcaacaacctgaaaaacaaactggaagaaaaagcgaacaaagcgatgatcaacatcaacatcttcatgcgtgaatcttctcgttctttcctggttaaccagatgatcaacgaagcgaaaaaacagctgctggaattcgacacccagtctaaaaacatcctgatgcagtacatcaaagcgaactctaaattcatcggtatcaccgaactgaaaaaactggaatctaaaatcaacaaagttttctctaccccgatcccgttctcttactctaaaaacctggactgctgggttgacaacgaagaagacatcgacgttatcctgaaaaaatctaccatcctgaacctggacatcaacaacgacatcatctctgacatctctggtttcaactcttctgttatcacctacccggacgcgcagctggttccgggtatcaacggtaaagcgatccacctggttaacaacgaatcttctgaagttatcgttcacaaagcgatggacatcgaatacaacgacatgttcaacaacttcaccgtttctttctggctgcgtgttccgaaagtttctgcgtgccacctggaacagtacggtaccaacgaatactctatcatctcttctatgaaaaaacactctctgtctatcggttctggttggtctgtttctctgaaaggtaacaacctgatctggaccctgaaagactctgcgggtgaagttcgtcagatcaccttccgtgacctgccggacaaattcaacgcgtacctggcgaacaaatgggttttcatcaccatcaccaacgaccgtctgtgctctgcgaacctgtacatcaacggtgttctgatgggttctgcggaaatcaccggtctgggtgcgatccgtgaagacaacaacatcaccctgaaactggaccgttgcaacaacaacaaccagtacgtttctatcgacaaattccgtatcttctgcaaagcgctgaacccgaaagaaatcgaaaaactgtacacctcttacctgtctatcaccttcctgcgtgacttctggggtaacccgctgcgttacgacaccgaatactacctgatcccggttgcgtcttcttctaaagacgttcagctgaaaaacatcaccgactacatgtacctgaccaacgcgccgtgctacaccaacggtaaactgaacatctactaccgtcgtctgtacaacggtctgaaattcatcatcaaacgttacaccccgaacaacgaaatcgactgcttcgttaaatctggtgacttcatcaaactgtacgtttcttacaacaacaacgaacacatcgttggttacccgaaagacggtaacgcgttcaacaacctggaccgtatcctgcgtgttggttacaacgcgccgggtatcccgctgtacaaaaaaatggaagcggttaaactgcgtgacctgaaaacctactctgttcagctgaaactgtacgacgacaaaaacgcgtctctgggtctggttggtacccacaacggtcagatcggtaacgacccgaaccgtgacatcctgatcgcgtctaactggtacttcaaccacctgaaagacaaaatcctgggttgcgactggtacttcgttccgaccgacgaaggttggaccaacgactaaaagcttgatccggctgctaacaaagcccgaaaggaagctgagttggctgctgccaccgctgagcaataactagcataaccccttggggcctctaaacgggtcttgaggggttttttgctgaaaggaggaactatatccggatctggcgtaatagcgaagaggcccgcaccgatcgcccttcccaacagttgcgcagcctgaatggcgaatgggacgcgccctgtagcggcgcattaagcgcggcgggtgtggtggttacgcgcagcgtgaccgctacacttgccagcgccctagcgcccgctcctttcgctttcttcccttcctttctcgccacgttcgccggctttccccgtcaagctctaaatcgggggctccctttagggttccgatttagtgctttacggcacctcgaccccaaaaaacttgattagggtgatggttcacgtagtgggccatcgccctgatagacggtttttcgccctttgacgttggagtccacgttctttaatagtggactcttgttccaaactggaacaacactcaaccctatctcggtctattcttttgatttataagggattttgccgatttcggcctattggttaaaaaatgagctgatttaacaaaaatttaacgcgaattttaacaaaatattaacgcttacaatttaggtggcacttttcggggaaatgtgcgcggaacccctatttgtttatttttctaaatacattcaaatatgtatccgctcatgagacaataaccctgataaatgcttcaataatattgaaaaaggaagagtatgagtattcaacatttccgtgtcgcccttattcccttttttgcggcattttgccttcctgtttttgctcacccagaaacgctggtgaaagtaaaagatgctgaagatcagttgggtgcacgagtgggttacatcgaactggatctcaacagcggtaagatccttgagagttttcgccccgaagaacgttttccaatgatgagcacttttaaagttctgctatgtggcgcggtattatcccgtattgacgccgggcaagagcaactcggtcgccgcatacactattctcagaatgacttggttgagtactcaccagtcacagaaaagcatcttacggatggcatgacagtaagagaattatgcagtgctgccataaccatgagtgataacactgcggccaacttacttctgacaacgatcggaggaccgaaggagctaaccgcttttttgcacaacatgggggatcatgtaactcgccttgatcgttgggaaccggagctgaatgaagccataccaaacgacgagcgtgacaccacgatgcctgtagcaatggcaacaacgttgcgcaaactattaactggcgaactacttactctagcttcccggcaacaattaatagactggatggaggcggataaagttgcaggaccacttctgcgctcggcccttccggctggctggtttattgctgataaatctggagccggtgagcgtgggtctcgcggtatcattgcagcactggggccagatggtaagccctcccgtatcgtagttatctacacgacggggagtcaggcaactatggatgaacgaaatagacagatcgctgagataggtgcctcactgattaagcattggtaactgtcagaccaagtttactcatatatactttagattgatttaaaacttcatttttaatttaaaaggatctaggtgaagatcctttttgataatctcatgaccaaaatcccttaacgtgagttttcgttccactgagcgtcagaccccgtagaaaagatcaaaggatcttcttgagatcctttttttctgcgcgtaatctgctgcttgcaaacaaaaaaaccaccgctaccagcggtggtttgtttgccggatcaagagctaccaactctttttccgaaggtaactggcttcagcagagcgcagataccaaatactgttcttctagtgtagccgtagttaggccaccacttcaagaactctgtagcaccgcctacatacctcgctctgctaatcctgttaccagtggctgctgccagtggcgataagtcgtgtcttaccgggttggactcaagacgatagttaccggataaggcgcagcggtcgggctgaacggggggttcgtgcacacagcccagcttggagcgaacgacctacaccgaactgagatacctacagcgtgagctatgagaaagcgccacgcttcccgaagggagaaaggcggacaggtatccggtaagcggcagggtcggaacaggagagcgcacgagggagcttccagggggaaacgcctggtatctttatagtcctgtcgggtttcgccacctctgacttgagcgtcgatttttgtgatgctcgtcaggggggcggagcctatggaaaaacgccagcaacgcggcctttttacggttcctggccttttgctggccttttgctcacatgttctttcctgcgttatcccctgattctgtggataaccgtattaccgcctttgagtgagctgataccgctcgccgcagccgaacgaccgagcgcagcgagtcagtgagcgaggaagcggaagagcgcccaatacgcaaaccgcctctccccgcgcgttggccgattcattaatgcag